European Patent Application EP 4 741 420 A1, published May 13, 2026. Title: GLP (Glucagon Like Peptide) 유사체를 유효성분으로 포함하는 비만 예방 또는 치료용 약학적 조성물. Applicant: 주식회사 휴온스랩. Application KR. The sequence listing filed with the application follows.

SEQUENCE LISTING (9 sequences)

SEQ ID NO: 1 - protein, 35 aa, synthetic construct
HGEGTFTSDLSTYLDALAARDFINWLIQTKITDKK

SEQ ID NO: 2 - protein, 33 aa, synthetic construct
HGEGTFTSDLSTYLDALAARDFINWLIQTKITD

SEQ ID NO: 3 - protein, 35 aa, synthetic construct; identical to SEQ ID NO: 1

SEQ ID NO: 4 - protein, 35 aa, synthetic construct; identical to SEQ ID NO: 1

SEQ ID NO: 5 - protein, 37 aa, synthetic construct
HAIBEGTFTSDLSTYLDALAARDFINWLIQTKITDKK

SEQ ID NO: 6 - protein, 37 aa, synthetic construct; identical to SEQ ID NO: 5

SEQ ID NO: 7 - protein, 37 aa, synthetic construct; identical to SEQ ID NO: 5

SEQ ID NO: 8 - protein, 35 aa, synthetic construct
HGEGTFTSDLSTYLDALAACDFINWLIQTKITDKK

SEQ ID NO: 9 - protein, 37 aa, synthetic construct
HAIBEGTFTSDLSTYLDALAARDFIKFAWLIQTKITD